European Patent Specification EP 3 859 056 B1, published December 25, 2024. Title: A method for producing protein fibers. Applicant: Spiber Inc. The sequence listing filed with the application follows.

SEQUENCE LISTING (62 sequences)

SEQ ID NO: 1 - protein, 50 aa, Araneus diadematus
SGCDVLVQALLEVVSALVSILGSSSIGQINYGASAQYTQMVGQSVAQALA

SEQ ID NO: 2 - protein, 30 aa, Araneus diadematus
SGCDVLVQALLEVVSALVSILGSSSIGQIN

SEQ ID NO: 3 - protein, 21 aa, Araneus diadematus
SGCDVLVQALLEVVSALVSIL

SEQ ID NO: 4 - protein, 1154 aa, Artificial Sequence
  recombinant spider silk protein ADF3KaiLargeNRSH1
MHHHHHHHHHHSSGSSLEVLFQGPARAGSGQQGPGQQGPGQQGPGQQGPYGPGASAAAAAAGGYGPGSGQQGPSQQGPGQQGPGGQGPYGPGASAAAAAAGGYGPGSGQQGPGGQGPYGPGSSAAAAAAGGNGPGSGQQGAGQQGPGQQGPGASAAAAAAGGYGPGSGQQGPGQQGPGGQGPYGPGASAAAAAAGGYGPGSGQGPGQQGPGGQGPYGPGASAAAAAAGGYGPGSGQQGPGQQGPGQQGPGGQGPYGPGASAAAAAAGGYGPGYGQQGPGQQGPGGQGPYGPGASAASAASGGYGPGSGQQGPGQQGPGGQGPYGPGASAAAAAAGGYGPGSGQQGPGQQGPGQQGPGQQGPGGQGPYGPGASAAAAAAGGYGPGSGQQGPGQQGPGQQGPGQQGPGQQGPGQQGPGQQGPGQQGPGQQGPGGQGAYGPGASAAAGAAGGYGPGSGQQGPGQQGPGQQGPGQQGPGQQGPGQQGPGQQGPGQQGPYGPGASAAAAAAGGYGPGSGQQGPGQQGPGQQGPGGQGPYGPGAASAAVSVSRARAGSGQQGPGQQGPGQQGPGQQGPYGPGASAAAAAAGGYGPGSGQQGPSQQGPGQQGPGGQGPYGPGASAAAAAAGGYGPGSGQQGPGGQGPYGPGSSAAAAAAGGNGPGSGQQGAGQQGPGQQGPGASAAAAAAGGYGPGSGQQGPGQQGPGGQGPYGPGASAAAAAAGGYGPGSGQGPGQQGPGGQGPYGPGASAAAAAAGGYGPGSGQQGPGQQGPGQQGPGGQGPYGPGASAAAAAAGGYGPGYGQQGPGQQGPGGQGPYGPGASAASAASGGYGPGSGQQGPGQQGPGGQGPYGPGASAAAAAAGGYGPGSGQQGPGQQGPGQQGPGQQGPGGQGPYGPGASAAAAAAGGYGPGSGQQGPGQQGPGQQGPGQQGPGQQGPGQQGPGQQGPGQQGPGQQGPGGQGAYGPGASAAAGAAGGYGPGSGQQGPGQQGPGQQGPGQQGPGQQGPGQQGPGQQGPGQQGPYGPGASAAAAAAGGYGPGSGQQGPGQQGPGQQGPGGQGPYGPGAASAAVSVGGYGPQSSSVPVASAVASRLSSPAASSRVSSAVSSLVSSGPTKHAALSNTISSVVSQVSASNPGLSGCDVLVQALLEVVSALVSIL

SEQ ID NO: 5 - protein, 24 aa, Artificial Sequence
  His tag and start codon
MHHHHHHHHHHSSGSSLEVLFQGP

SEQ ID NO: 6 - protein, 597 aa, Artificial Sequence
  Met-PRT380
MGPGQQGPYGPGASAAAAAGQNGPGSGQQGPGQSAAAAAGQYGPGQQGPGQQGPGSSAAAAAGPGQYGPGQQGPSASAAAAAGPGSGQQGPGASAAAAAGQYGPGQQGPGQQGPGSSAAAAAGQYGSGPGQQGPYGSAAAAAGPGSGQYGQGPYGPGASAAAAAGPGQYGPGQQGPSASAAAAAGSGQQGPGQYGPYASAAAAAGQYGSGPGQQGPYGPGQSAAAAAGSGQQGPGQQGPYASAAAAAGPGQQGPYGPGSSAAAAAGQYGYGPGQQGPYGPGASAAAAAGQNGPGSGQYGPGQQGPGQSAAAAAGPGQQGPYGPGASAAAAAGQYGPGQQGPGQYGPGSSAAAAAGPGQQGPYGPGSSAAAAAGQYGPGQQGPYGPGQSAAAAAGQYQQGPGQQGPYGPGASAAAAAGPGQQGPYGPGASAAAAAGPGQYGPGQQGPSASAAAAAGQYGSGPGQYGPYGPGQSAAAAAGPGSGQQGQGPYGPGASAAAAAGQYGPGQQGPYGPGQSAAAAAGPGSGQYGPGASAAAAAGQNGPGSGQYGPGQQGPGQSAAAAAGQYQQGPGQQGPYGPGASAAAAAGPGSGQQGPGAS

SEQ ID NO: 7 - protein, 590 aa, Artificial Sequence
  Met-PRT410
MGPGQQGPYGPGASAAAAAGQNGPGSGQQGPGQSGQYGPGQQGPGQQGPGSSAAAAAGPGQYGPGQQGPSASAAAAAGPGSGQQGPGASGQYGPGQQGPGQQGPGSSAAAAAGQYGSGPGQQGPYGSAAAAAGPGSGQYGQGPYGPGASGPGQYGPGQQGPSASAAAAAGSGQQGPGQYGPYASAAAAAGQYGSGPGQQGPYGPGQSGSGQQGPGQQGPYASAAAAAGPGQQGPYGPGSSAAAAAGQYGYGPGQQGPYGPGASGQNGPGSGQYGPGQQGPGQSAAAAAGPGQQGPYGPGASAAAAAGQYGPGQQGPGQYGPGSSGPGQQGPYGPGSSAAAAAGQYGPGQQGPYGPGQSAAAAAGQYQQGPGQQGPYGPGASGPGQQGPYGPGASAAAAAGPGQYGPGQQGPSASAAAAAGQYGSGPGQYGPYGPGQSGPGSGQQGQGPYGPGASAAAAAGQYGPGQQGPYGPGQSAAAAAGPGSGQYGPGASGQNGPGSGQYGPGQQGPGQSAAAAAGQYQQGPGQQGPYGPGASAAAAAGQYGSGPGQQGPYGPGQSGSGQQGPGQQGPYASAAAAAGPGSGQQGPGAS

SEQ ID NO: 8 - protein, 565 aa, Artificial Sequence
  Met-PRT468
MGPGQQGPYGPGASAAAAAAAGSNGPGSGQQGPGQSGQYGPGQQGPGQQGPGSSAAAAAAAGPGQYGPGQQGPSASAAAAAAAGPGSGQQGPGASGQYGPGQQGPGQQGPGSSAAAAAAAGSYGSGPGQQGPYGSAAAAAAAGPGSGQYGQGPYGPGASGPGQYGPGQQGPSASAAAAAAAGSGQQGPGQYGPYASAAAAAAAGSYGSGPGQQGPYGPGQSGSGQQGPGQQGPYASAAAAAAAGPGQQGPYGPGSSAAAAAAAGSYGYGPGQQGPYGPGASGQNGPGSGQYGPGQQGPGPSAAAAAAAGPGQQGPYGPGASAAAAAAAGSYGPGQQGPGQYGPGSSGPGQQGPYGPGSSAAAAAAAGSYGPGQQGPYGPGPSAAAAAAAGSYQQGPGQQGPYGPGASGPGQQGPYGPGASAAAAAAAGPGQYGPGQQGPSASAAAAAAAGSYGSGPGQYGPYGPGQSGPGSGQQGQGPYGPGASAAAAAAAGSYGPGQQGPYGPGPSAAAAAAAGPGSGQYGPGASGQNGPGSGQYGPGQQGPGPSAAAAAAAGPGSGQQGPGAS

SEQ ID NO: 9 - protein, 2364 aa, Artificial Sequence
  Met-PRT799
MGPGQQGPYGPGASAAAAAGQNGPGSGQQGPGQSGQYGPGQQGPGQQGPGSSAAAAAGPGQYGPGQQGPSASAAAAAGPGSGQQGPGASGQYGPGQQGPGQQGPGSSAAAAAGQYGSGPGQQGPYGSAAAAAGPGSGQYGQGPYGPGASGPGQYGPGQQGPSASAAAAAGSGQQGPGQYGPYASAAAAAGQYGSGPGQQGPYGPGQSGSGQQGPGQQGPYASAAAAAGPGQQGPYGPGSSAAAAAGQYGYGPGQQGPYGPGASGQNGPGSGQYGPGQQGPGQSAAAAAGPGQQGPYGPGASAAAAAGQYGPGQQGPGQYGPGSSGPGQQGPYGPGSSAAAAAGQYGPGQQGPYGPGQSAAAAAGQYQQGPGQQGPYGPGASGPGQQGPYGPGASAAAAAGPGQYGPGQQGPSASAAAAAGQYGSGPGQYGPYGPGQSGPGSGQQGQGPYGPGASAAAAAGQYGPGQQGPYGPGQSAAAAAGPGSGQYGPGASGQNGPGSGQYGPGQQGPGQSAAAAAGQYQQGPGQQGPYGPGASAAAAAGQYGSGPGQQGPYGPGQSGSGQQGPGQQGPYASAAAAAGPGSGQQGPGASGQQGPYGPGASAAAAAGQNGPGSGQQGPGQSGQYGPGQQGPGQQGPGSSAAAAAGPGQYGPGQQGPSASAAAAAGPGSGQQGPGASGQYGPGQQGPGQQGPGSSAAAAAGQYGSGPGQQGPYGSAAAAAGPGSGQYGQGPYGPGASGPGQYGPGQQGPSASAAAAAGSGQQGPGQYGPYASAAAAAGQYGSGPGQQGPYGPGQSGSGQQGPGQQGPYASAAAAAGPGQQGPYGPGSSAAAAAGQYGYGPGQQGPYGPGASGQNGPGSGQYGPGQQGPGQSAAAAAGPGQQGPYGPGASAAAAAGQYGPGQQGPGQYGPGSSGPGQQGPYGPGSSAAAAAGQYGPGQQGPYGPGQSAAAAAGQYQQGPGQQGPYGPGASGPGQQGPYGPGASAAAAAGPGQYGPGQQGPSASAAAAAGQYGSGPGQYGPYGPGQSGPGSGQQGQGPYGPGASAAAAAGQYGPGQQGPYGPGQSAAAAAGPGSGQYGPGASGQNGPGSGQYGPGQQGPGQSAAAAAGQYQQGPGQQGPYGPGASAAAAAGQYGSGPGQQGPYGPGQSGSGQQGPGQQGPYASAAAAAGPGSGQQGPGASGQQGPYGPGASAAAAAGQNGPGSGQQGPGQSGQYGPGQQGPGQQGPGSSAAAAAGPGQYGPGQQGPSASAAAAAGPGSGQQGPGASGQYGPGQQGPGQQGPGSSAAAAAGQYGSGPGQQGPYGSAAAAAGPGSGQYGQGPYGPGASGPGQYGPGQQGPSASAAAAAGSGQQGPGQYGPYASAAAAAGQYGSGPGQQGPYGPGQSGSGQQGPGQQGPYASAAAAAGPGQQGPYGPGSSAAAAAGQYGYGPGQQGPYGPGASGQNGPGSGQYGPGQQGPGQSAAAAAGPGQQGPYGPGASAAAAAGQYGPGQQGPGQYGPGSSGPGQQGPYGPGSSAAAAAGQYGPGQQGPYGPGQSAAAAAGQYQQGPGQQGPYGPGASGPGQQGPYGPGASAAAAAGPGQYGPGQQGPSASAAAAAGQYGSGPGQYGPYGPGQSGPGSGQQGQGPYGPGASAAAAAGQYGPGQQGPYGPGQSAAAAAGPGSGQYGPGASGQNGPGSGQYGPGQQGPGQSAAAAAGQYQQGPGQQGPYGPGASAAAAAGQYGSGPGQQGPYGPGQSGSGQQGPGQQGPYASAAAAAGPGSGQQGPGASGQQGPYGPGASAAAAAGQNGPGSGQQGPGQSGQYGPGQQGPGQQGPGSSAAAAAGPGQYGPGQQGPSASAAAAAGPGSGQQGPGASGQYGPGQQGPGQQGPGSSAAAAAGQYGSGPGQQGPYGSAAAAAGPGSGQYGQGPYGPGASGPGQYGPGQQGPSASAAAAAGSGQQGPGQYGPYASAAAAAGQYGSGPGQQGPYGPGQSGSGQQGPGQQGPYASAAAAAGPGQQGPYGPGSSAAAAAGQYGYGPGQQGPYGPGASGQNGPGSGQYGPGQQGPGQSAAAAAGPGQQGPYGPGASAAAAAGQYGPGQQGPGQYGPGSSGPGQQGPYGPGSSAAAAAGQYGPGQQGPYGPGQSAAAAAGQYQQGPGQQGPYGPGASGPGQQGPYGPGASAAAAAGPGQYGPGQQGPSASAAAAAGQYGSGPGQYGPYGPGQSGPGSGQQGQGPYGPGASAAAAAGQYGPGQQGPYGPGQSAAAAAGPGSGQYGPGASGQNGPGSGQYGPGQQGPGQSAAAAAGQYQQGPGQQGPYGPGASAAAAAGQYGSGPGQQGPYGPGQSGSGQQGPGQQGPYASAAAAAGPGSGQQGSSVDKLAAALEHHHHHH

SEQ ID NO: 10 - protein, 597 aa, Artificial Sequence
  Met-PRT313
MGPGGQGPYGPGASAAAAAGGNGPGSGQQGPGGSAAAAAGGYGPGGQGPGQQGPGSSAAAAAGPGGYGPGGQGPSASAAAAAGPGSGQQGPGASAAAAAGGYGPGGQGPGQQGPGSSAAAAAGGYGSGPGQQGPYGSAAAAAGPGSGGYGQGPYGPGASAAAAAGPGGYGPGGQGPSASAAAAAGSGQQGPGGYGPYASAAAAAGGYGSGPGQQGPYGPGGSAAAAAGSGQQGPGQQGPYASAAAAAGPGGQGPYGPGSSAAAAAGGYGYGPGGQGPYGPGASAAAAAGGNGPGSGGYGPGQQGPGGSAAAAAGPGGQGPYGPGASAAAAAGGYGPGGQGPGGYGPGSSAAAAAGPGGQGPYGPGSSAAAAAGGYGPGQQGPYGPGGSAAAAAGGYQQGPGGQGPYGPGASAAAAAGPGGQGPYGPGASAAAAAGPGGYGPGGQGPSASAAAAAGGYGSGPGGYGPYGPGGSAAAAAGPGSGQQGQGPYGPGASAAAAAGGYGPGQQGPYGPGGSAAAAAGPGSGGYGPGASAAAAAGGNGPGSGGYGPGQQGPGGSAAAAAGGYQQGPGGQGPYGPGASAAAAAGPGSGQQGPGAS

SEQ ID NO: 11 - protein, 601 aa, Artificial Sequence
  PRT410
MHHHHHHSSGSSGPGQQGPYGPGASAAAAAGQNGPGSGQQGPGQSGQYGPGQQGPGQQGPGSSAAAAAGPGQYGPGQQGPSASAAAAAGPGSGQQGPGASGQYGPGQQGPGQQGPGSSAAAAAGQYGSGPGQQGPYGSAAAAAGPGSGQYGQGPYGPGASGPGQYGPGQQGPSASAAAAAGSGQQGPGQYGPYASAAAAAGQYGSGPGQQGPYGPGQSGSGQQGPGQQGPYASAAAAAGPGQQGPYGPGSSAAAAAGQYGYGPGQQGPYGPGASGQNGPGSGQYGPGQQGPGQSAAAAAGPGQQGPYGPGASAAAAAGQYGPGQQGPGQYGPGSSGPGQQGPYGPGSSAAAAAGQYGPGQQGPYGPGQSAAAAAGQYQQGPGQQGPYGPGASGPGQQGPYGPGASAAAAAGPGQYGPGQQGPSASAAAAAGQYGSGPGQYGPYGPGQSGPGSGQQGQGPYGPGASAAAAAGQYGPGQQGPYGPGQSAAAAAGPGSGQYGPGASGQNGPGSGQYGPGQQGPGQSAAAAAGQYQQGPGQQGPYGPGASAAAAAGQYGSGPGQQGPYGPGQSGSGQQGPGQQGPYASAAAAAGPGSGQQGPGAS

SEQ ID NO: 12 - protein, 12 aa, Artificial Sequence
  HisTag
MHHHHHHSSGSS

SEQ ID NO: 13 - protein, 608 aa, Artificial Sequence
  PRT380
MHHHHHHSSGSSGPGQQGPYGPGASAAAAAGQNGPGSGQQGPGQSAAAAAGQYGPGQQGPGQQGPGSSAAAAAGPGQYGPGQQGPSASAAAAAGPGSGQQGPGASAAAAAGQYGPGQQGPGQQGPGSSAAAAAGQYGSGPGQQGPYGSAAAAAGPGSGQYGQGPYGPGASAAAAAGPGQYGPGQQGPSASAAAAAGSGQQGPGQYGPYASAAAAAGQYGSGPGQQGPYGPGQSAAAAAGSGQQGPGQQGPYASAAAAAGPGQQGPYGPGSSAAAAAGQYGYGPGQQGPYGPGASAAAAAGQNGPGSGQYGPGQQGPGQSAAAAAGPGQQGPYGPGASAAAAAGQYGPGQQGPGQYGPGSSAAAAAGPGQQGPYGPGSSAAAAAGQYGPGQQGPYGPGQSAAAAAGQYQQGPGQQGPYGPGASAAAAAGPGQQGPYGPGASAAAAAGPGQYGPGQQGPSASAAAAAGQYGSGPGQYGPYGPGQSAAAAAGPGSGQQGQGPYGPGASAAAAAGQYGPGQQGPYGPGQSAAAAAGPGSGQYGPGASAAAAAGQNGPGSGQYGPGQQGPGQSAAAAAGQYQQGPGQQGPYGPGASAAAAAGPGSGQQGPGAS

SEQ ID NO: 14 - protein, 576 aa, Artificial Sequence
  PRT468
MHHHHHHSSGSSGPGQQGPYGPGASAAAAAAAGSNGPGSGQQGPGQSGQYGPGQQGPGQQGPGSSAAAAAAAGPGQYGPGQQGPSASAAAAAAAGPGSGQQGPGASGQYGPGQQGPGQQGPGSSAAAAAAAGSYGSGPGQQGPYGSAAAAAAAGPGSGQYGQGPYGPGASGPGQYGPGQQGPSASAAAAAAAGSGQQGPGQYGPYASAAAAAAAGSYGSGPGQQGPYGPGQSGSGQQGPGQQGPYASAAAAAAAGPGQQGPYGPGSSAAAAAAAGSYGYGPGQQGPYGPGASGQNGPGSGQYGPGQQGPGPSAAAAAAAGPGQQGPYGPGASAAAAAAAGSYGPGQQGPGQYGPGSSGPGQQGPYGPGSSAAAAAAAGSYGPGQQGPYGPGPSAAAAAAAGSYQQGPGQQGPYGPGASGPGQQGPYGPGASAAAAAAAGPGQYGPGQQGPSASAAAAAAAGSYGSGPGQYGPYGPGQSGPGSGQQGQGPYGPGASAAAAAAAGSYGPGQQGPYGPGPSAAAAAAAGPGSGQYGPGASGQNGPGSGQYGPGQQGPGPSAAAAAAAGPGSGQQGPGAS

SEQ ID NO: 15 - protein, 2375 aa, Artificial Sequence
  PRT799
MHHHHHHSSGSSGPGQQGPYGPGASAAAAAGQNGPGSGQQGPGQSGQYGPGQQGPGQQGPGSSAAAAAGPGQYGPGQQGPSASAAAAAGPGSGQQGPGASGQYGPGQQGPGQQGPGSSAAAAAGQYGSGPGQQGPYGSAAAAAGPGSGQYGQGPYGPGASGPGQYGPGQQGPSASAAAAAGSGQQGPGQYGPYASAAAAAGQYGSGPGQQGPYGPGQSGSGQQGPGQQGPYASAAAAAGPGQQGPYGPGSSAAAAAGQYGYGPGQQGPYGPGASGQNGPGSGQYGPGQQGPGQSAAAAAGPGQQGPYGPGASAAAAAGQYGPGQQGPGQYGPGSSGPGQQGPYGPGSSAAAAAGQYGPGQQGPYGPGQSAAAAAGQYQQGPGQQGPYGPGASGPGQQGPYGPGASAAAAAGPGQYGPGQQGPSASAAAAAGQYGSGPGQYGPYGPGQSGPGSGQQGQGPYGPGASAAAAAGQYGPGQQGPYGPGQSAAAAAGPGSGQYGPGASGQNGPGSGQYGPGQQGPGQSAAAAAGQYQQGPGQQGPYGPGASAAAAAGQYGSGPGQQGPYGPGQSGSGQQGPGQQGPYASAAAAAGPGSGQQGPGASGQQGPYGPGASAAAAAGQNGPGSGQQGPGQSGQYGPGQQGPGQQGPGSSAAAAAGPGQYGPGQQGPSASAAAAAGPGSGQQGPGASGQYGPGQQGPGQQGPGSSAAAAAGQYGSGPGQQGPYGSAAAAAGPGSGQYGQGPYGPGASGPGQYGPGQQGPSASAAAAAGSGQQGPGQYGPYASAAAAAGQYGSGPGQQGPYGPGQSGSGQQGPGQQGPYASAAAAAGPGQQGPYGPGSSAAAAAGQYGYGPGQQGPYGPGASGQNGPGSGQYGPGQQGPGQSAAAAAGPGQQGPYGPGASAAAAAGQYGPGQQGPGQYGPGSSGPGQQGPYGPGSSAAAAAGQYGPGQQGPYGPGQSAAAAAGQYQQGPGQQGPYGPGASGPGQQGPYGPGASAAAAAGPGQYGPGQQGPSASAAAAAGQYGSGPGQYGPYGPGQSGPGSGQQGQGPYGPGASAAAAAGQYGPGQQGPYGPGQSAAAAAGPGSGQYGPGASGQNGPGSGQYGPGQQGPGQSAAAAAGQYQQGPGQQGPYGPGASAAAAAGQYGSGPGQQGPYGPGQSGSGQQGPGQQGPYASAAAAAGPGSGQQGPGASGQQGPYGPGASAAAAAGQNGPGSGQQGPGQSGQYGPGQQGPGQQGPGSSAAAAAGPGQYGPGQQGPSASAAAAAGPGSGQQGPGASGQYGPGQQGPGQQGPGSSAAAAAGQYGSGPGQQGPYGSAAAAAGPGSGQYGQGPYGPGASGPGQYGPGQQGPSASAAAAAGSGQQGPGQYGPYASAAAAAGQYGSGPGQQGPYGPGQSGSGQQGPGQQGPYASAAAAAGPGQQGPYGPGSSAAAAAGQYGYGPGQQGPYGPGASGQNGPGSGQYGPGQQGPGQSAAAAAGPGQQGPYGPGASAAAAAGQYGPGQQGPGQYGPGSSGPGQQGPYGPGSSAAAAAGQYGPGQQGPYGPGQSAAAAAGQYQQGPGQQGPYGPGASGPGQQGPYGPGASAAAAAGPGQYGPGQQGPSASAAAAAGQYGSGPGQYGPYGPGQSGPGSGQQGQGPYGPGASAAAAAGQYGPGQQGPYGPGQSAAAAAGPGSGQYGPGASGQNGPGSGQYGPGQQGPGQSAAAAAGQYQQGPGQQGPYGPGASAAAAAGQYGSGPGQQGPYGPGQSGSGQQGPGQQGPYASAAAAAGPGSGQQGPGASGQQGPYGPGASAAAAAGQNGPGSGQQGPGQSGQYGPGQQGPGQQGPGSSAAAAAGPGQYGPGQQGPSASAAAAAGPGSGQQGPGASGQYGPGQQGPGQQGPGSSAAAAAGQYGSGPGQQGPYGSAAAAAGPGSGQYGQGPYGPGASGPGQYGPGQQGPSASAAAAAGSGQQGPGQYGPYASAAAAAGQYGSGPGQQGPYGPGQSGSGQQGPGQQGPYASAAAAAGPGQQGPYGPGSSAAAAAGQYGYGPGQQGPYGPGASGQNGPGSGQYGPGQQGPGQSAAAAAGPGQQGPYGPGASAAAAAGQYGPGQQGPGQYGPGSSGPGQQGPYGPGSSAAAAAGQYGPGQQGPYGPGQSAAAAAGQYQQGPGQQGPYGPGASGPGQQGPYGPGASAAAAAGPGQYGPGQQGPSASAAAAAGQYGSGPGQYGPYGPGQSGPGSGQQGQGPYGPGASAAAAAGQYGPGQQGPYGPGQSAAAAAGPGSGQYGPGASGQNGPGSGQYGPGQQGPGQSAAAAAGQYQQGPGQQGPYGPGASAAAAAGQYGSGPGQQGPYGPGQSGSGQQGPGQQGPYASAAAAAGPGSGQQGSSVDKLAAALEHHHHHH

SEQ ID NO: 16 - protein, 608 aa, Artificial Sequence
  PRT313
MHHHHHHSSGSSGPGGQGPYGPGASAAAAAGGNGPGSGQQGPGGSAAAAAGGYGPGGQGPGQQGPGSSAAAAAGPGGYGPGGQGPSASAAAAAGPGSGQQGPGASAAAAAGGYGPGGQGPGQQGPGSSAAAAAGGYGSGPGQQGPYGSAAAAAGPGSGGYGQGPYGPGASAAAAAGPGGYGPGGQGPSASAAAAAGSGQQGPGGYGPYASAAAAAGGYGSGPGQQGPYGPGGSAAAAAGSGQQGPGQQGPYASAAAAAGPGGQGPYGPGSSAAAAAGGYGYGPGGQGPYGPGASAAAAAGGNGPGSGGYGPGQQGPGGSAAAAAGPGGQGPYGPGASAAAAAGGYGPGGQGPGGYGPGSSAAAAAGPGGQGPYGPGSSAAAAAGGYGPGQQGPYGPGGSAAAAAGGYQQGPGGQGPYGPGASAAAAAGPGGQGPYGPGASAAAAAGPGGYGPGGQGPSASAAAAAGGYGSGPGGYGPYGPGGSAAAAAGPGSGQQGQGPYGPGASAAAAAGGYGPGQQGPYGPGGSAAAAAGPGSGGYGPGASAAAAAGGNGPGSGGYGPGQQGPGGSAAAAAGGYQQGPGGQGPYGPGASAAAAAGPGSGQQGPGAS

SEQ ID NO: 17 - protein, 601 aa, Artificial Sequence
  PRT399
MHHHHHHSSGSSGPGGQGPYGPGASAAAAAGGNGPGSGQQGPGGSGGYGPGGQGPGQQGPGSSAAAAAGPGGYGPGGQGPSASAAAAAGPGSGQQGPGASGGYGPGGQGPGQQGPGSSAAAAAGGYGSGPGQQGPYGSAAAAAGPGSGGYGQGPYGPGASGPGGYGPGGQGPSASAAAAAGSGQQGPGGYGPYASAAAAAGGYGSGPGQQGPYGPGGSGSGQQGPGQQGPYASAAAAAGPGGQGPYGPGSSAAAAAGGYGYGPGGQGPYGPGASGGNGPGSGGYGPGQQGPGGSAAAAAGPGGQGPYGPGASAAAAAGGYGPGGQGPGGYGPGSSGPGGQGPYGPGSSAAAAAGGYGPGQQGPYGPGGSAAAAAGGYQQGPGGQGPYGPGASGPGGQGPYGPGASAAAAAGPGGYGPGGQGPSASAAAAAGGYGSGPGGYGPYGPGGSGPGSGQQGQGPYGPGASAAAAAGGYGPGQQGPYGPGGSAAAAAGPGSGGYGPGASGGNGPGSGGYGPGQQGPGGSAAAAAGGYQQGPGGQGPYGPGASAAAAAGGYGSGPGQQGPYGPGGSGSGQQGPGQQGPYASAAAAAGPGSGQQGPGAS

SEQ ID NO: 18 - protein, 590 aa, Artificial Sequence
  Met-PRT399
MGPGGQGPYGPGASAAAAAGGNGPGSGQQGPGGSGGYGPGGQGPGQQGPGSSAAAAAGPGGYGPGGQGPSASAAAAAGPGSGQQGPGASGGYGPGGQGPGQQGPGSSAAAAAGGYGSGPGQQGPYGSAAAAAGPGSGGYGQGPYGPGASGPGGYGPGGQGPSASAAAAAGSGQQGPGGYGPYASAAAAAGGYGSGPGQQGPYGPGGSGSGQQGPGQQGPYASAAAAAGPGGQGPYGPGSSAAAAAGGYGYGPGGQGPYGPGASGGNGPGSGGYGPGQQGPGGSAAAAAGPGGQGPYGPGASAAAAAGGYGPGGQGPGGYGPGSSGPGGQGPYGPGSSAAAAAGGYGPGQQGPYGPGGSAAAAAGGYQQGPGGQGPYGPGASGPGGQGPYGPGASAAAAAGPGGYGPGGQGPSASAAAAAGGYGSGPGGYGPYGPGGSGPGSGQQGQGPYGPGASAAAAAGGYGPGQQGPYGPGGSAAAAAGPGSGGYGPGASGGNGPGSGGYGPGQQGPGGSAAAAAGGYQQGPGGQGPYGPGASAAAAAGGYGSGPGQQGPYGPGGSGSGQQGPGQQGPYASAAAAAGPGSGQQGPGAS

SEQ ID NO: 19 - protein, 612 aa, Artificial Sequence
  Met-PRT720
MGPGQQGPYGPGASAAAAAGQNGPGSGQQGPGQSGQYGPGQQGPGQQGPGSSAAAAAGPGQYVLIGPGQQVLIGPSASAAAAAGPGSGQQGPGASGQYGPGQQGPGQQGPGSSAAAAAGSYGSVLIGPGQQVLIGPYGSAAAAAGPGSGQYGQGPYGPGASGPGQYGPGQQGPSASAAAAAGSGQQVLIGPGQYVLIGPYASAAAAAGQYGSGPGQQGPYGPGQSGSGQQGPGQQGPYASAAAAAGPGQQVLIGPYVLIGPGSSAAAAAGQYGYGPGQQGPYGPGASGQNGPGSGQYGPGQQGPGQSAAAAAGPGQQVLIGPYVLIGPGASAAAAAGQYGPGQQGPGQYGPGSSGPGQQGPYGPGSSAAAAAGSYGPGQQVLIGPYVLIGPGPSAAAAAGQYQQGPGQQGPYGPGASGPGQQGPYGPGASAAAAAGPGQYVLIGPGQQVLIGPSASAAAAAGQYGSGPGQYGPYGPGQSGPGSGQQGQGPYGPGASAAAAAGSYGPGQQVLIGPYVLIGPGPSAAAAAGPGSGQYGPGASGQNGPGSGQYGPGQQGPGQSAAAAAGQYQQVLIGPGQQGPYVLIGPGASAAAAAGPGSGQQVLIGPGASVLI

SEQ ID NO: 20 - protein, 592 aa, Artificial Sequence
  Met-PRT665
MGPGQQGPYGPGASAAAAAAAGSNGPGSGQQGPGQSGQYGPGQQGPGQQGPGSSAAAAAAAGPGQYVLIGPGQQGPSASAAAAAAAGPGSGQQGPGASGQYGPGQQGPGQQGPGSSAAAAAAAGSYGSVLIGPGQQGPYGSAAAAAAAGPGSGQYGQGPYGPGASGPGQYGPGQQGPSASAAAAAAAGSGQQVLIGPGQYGPYASAAAAAAAGSYGSGPGQQGPYGPGQSGSGQQGPGQQGPYASAAAAAAAGPGQQVLIGPYGPGSSAAAAAAAGSYGYGPGQQGPYGPGASGQNGPGSGQYGPGQQGPGPSAAAAAAAGPGQQVLIGPYGPGASAAAAAAAGSYGPGQQGPGQYGPGSSGPGQQGPYGPGSSAAAAAAAGSYGPGQQVLIGPYGPGPSAAAAAAAGSYQQGPGQQGPYGPGASGPGQQGPYGPGASAAAAAAAGPGQYVLIGPGQQGPSASAAAAAAAGSYGSGPGQYGPYGPGQSGPGSGQQGQGPYGPGASAAAAAAAGSYGPGQQVLIGPYGPGPSAAAAAAAGPGSGQYGPGASGQNGPGSGQYGPGQQGPGPSAAAAAAAGPGSGQQGPGASVLI

SEQ ID NO: 21 - protein, 619 aa, Artificial Sequence
  Met-PRT666
MGPGQQGPYGPGASAAAAAAAGSNGPGSGQQGPGQSGQYGPGQQGPGQQGPGSSAAAAAAAGPGQYVLIGPGQQVLIGPSASAAAAAAAGPGSGQQGPGASGQYGPGQQGPGQQGPGSSAAAAAAAGSYGSVLIGPGQQVLIGPYGSAAAAAAAGPGSGQYGQGPYGPGASGPGQYGPGQQGPSASAAAAAAAGSGQQVLIGPGQYVLIGPYASAAAAAAAGSYGSGPGQQGPYGPGQSGSGQQGPGQQGPYASAAAAAAAGPGQQVLIGPYVLIGPGSSAAAAAAAGSYGYGPGQQGPYGPGASGQNGPGSGQYGPGQQGPGPSAAAAAAAGPGQQVLIGPYVLIGPGASAAAAAAAGSYGPGQQGPGQYGPGSSGPGQQGPYGPGSSAAAAAAAGSYGPGQQVLIGPYVLIGPGPSAAAAAAAGSYQQGPGQQGPYGPGASGPGQQGPYGPGASAAAAAAAGPGQYVLIGPGQQVLIGPSASAAAAAAAGSYGSGPGQYGPYGPGQSGPGSGQQGQGPYGPGASAAAAAAAGSYGPGQQVLIGPYVLIGPGPSAAAAAAAGPGSGQYGPGASGQNGPGSGQYGPGQQGPGPSAAAAAAAGPGSGQQVLIGPGASVLI

SEQ ID NO: 22 - protein, 590 aa, Artificial Sequence; identical to SEQ ID NO: 7
  Met-PRT410

SEQ ID NO: 23 - protein, 565 aa, Artificial Sequence; identical to SEQ ID NO: 8
  Met-PRT468

SEQ ID NO: 24 - protein, 623 aa, Artificial Sequence
  PRT468
MHHHHHHSSGSSGPGQQGPYGPGASAAAAAGQNGPGSGQQGPGQSGQYGPGQQGPGQQGPGSSAAAAAGPGQYVLIGPGQQVLIGPSASAAAAAGPGSGQQGPGASGQYGPGQQGPGQQGPGSSAAAAAGSYGSVLIGPGQQVLIGPYGSAAAAAGPGSGQYGQGPYGPGASGPGQYGPGQQGPSASAAAAAGSGQQVLIGPGQYVLIGPYASAAAAAGQYGSGPGQQGPYGPGQSGSGQQGPGQQGPYASAAAAAGPGQQVLIGPYVLIGPGSSAAAAAGQYGYGPGQQGPYGPGASGQNGPGSGQYGPGQQGPGQSAAAAAGPGQQVLIGPYVLIGPGASAAAAAGQYGPGQQGPGQYGPGSSGPGQQGPYGPGSSAAAAAGSYGPGQQVLIGPYVLIGPGPSAAAAAGQYQQGPGQQGPYGPGASGPGQQGPYGPGASAAAAAGPGQYVLIGPGQQVLIGPSASAAAAAGQYGSGPGQYGPYGPGQSGPGSGQQGQGPYGPGASAAAAAGSYGPGQQVLIGPYVLIGPGPSAAAAAGPGSGQYGPGASGQNGPGSGQYGPGQQGPGQSAAAAAGQYQQVLIGPGQQGPYVLIGPGASAAAAAGPGSGQQVLIGPGASVLI

SEQ ID NO: 25 - protein, 603 aa, Artificial Sequence
  PRT665
MHHHHHHSSGSSGPGQQGPYGPGASAAAAAAAGSNGPGSGQQGPGQSGQYGPGQQGPGQQGPGSSAAAAAAAGPGQYVLIGPGQQGPSASAAAAAAAGPGSGQQGPGASGQYGPGQQGPGQQGPGSSAAAAAAAGSYGSVLIGPGQQGPYGSAAAAAAAGPGSGQYGQGPYGPGASGPGQYGPGQQGPSASAAAAAAAGSGQQVLIGPGQYGPYASAAAAAAAGSYGSGPGQQGPYGPGQSGSGQQGPGQQGPYASAAAAAAAGPGQQVLIGPYGPGSSAAAAAAAGSYGYGPGQQGPYGPGASGQNGPGSGQYGPGQQGPGPSAAAAAAAGPGQQVLIGPYGPGASAAAAAAAGSYGPGQQGPGQYGPGSSGPGQQGPYGPGSSAAAAAAAGSYGPGQQVLIGPYGPGPSAAAAAAAGSYQQGPGQQGPYGPGASGPGQQGPYGPGASAAAAAAAGPGQYVLIGPGQQGPSASAAAAAAAGSYGSGPGQYGPYGPGQSGPGSGQQGQGPYGPGASAAAAAAAGSYGPGQQVLIGPYGPGPSAAAAAAAGPGSGQYGPGASGQNGPGSGQYGPGQQGPGPSAAAAAAAGPGSGQQGPGASVLI

SEQ ID NO: 26 - protein, 630 aa, Artificial Sequence
  PRT666
MHHHHHHSSGSSGPGQQGPYGPGASAAAAAAAGSNGPGSGQQGPGQSGQYGPGQQGPGQQGPGSSAAAAAAAGPGQYVLIGPGQQVLIGPSASAAAAAAAGPGSGQQGPGASGQYGPGQQGPGQQGPGSSAAAAAAAGSYGSVLIGPGQQVLIGPYGSAAAAAAAGPGSGQYGQGPYGPGASGPGQYGPGQQGPSASAAAAAAAGSGQQVLIGPGQYVLIGPYASAAAAAAAGSYGSGPGQQGPYGPGQSGSGQQGPGQQGPYASAAAAAAAGPGQQVLIGPYVLIGPGSSAAAAAAAGSYGYGPGQQGPYGPGASGQNGPGSGQYGPGQQGPGPSAAAAAAAGPGQQVLIGPYVLIGPGASAAAAAAAGSYGPGQQGPGQYGPGSSGPGQQGPYGPGSSAAAAAAAGSYGPGQQVLIGPYVLIGPGPSAAAAAAAGSYQQGPGQQGPYGPGASGPGQQGPYGPGASAAAAAAAGPGQYVLIGPGQQVLIGPSASAAAAAAAGSYGSGPGQYGPYGPGQSGPGSGQQGQGPYGPGASAAAAAAAGSYGPGQQVLIGPYVLIGPGPSAAAAAAAGPGSGQYGPGASGQNGPGSGQYGPGQQGPGPSAAAAAAAGPGSGQQVLIGPGASVLI

SEQ ID NO: 27 - protein, 593 aa, Artificial Sequence
  M_PRT888
MGSSGPGVLGPYGPGASAAAAAGQNGPGSGVLGPGQSGQYGPGVLGPGVLGPGSSAAAAAGPGQYGPGVLGPSASAAAAAGPGSGVLGPGASGQYGPGVLGPGVLGPGSSAAAAAGQYGSGPGVLGPYGSAAAAAGPGSGQYGQGPYGPGASGPGQYGPGVLGPSASAAAAAGSGVLGPGQYGPYASAAAAAGQYGSGPGVLGPYGPGQSGSGVLGPGVLGPYASAAAAAGPGVLGPYGPGSSAAAAAGQYGYGPGVLGPYGPGASGQNGPGSGQYGPGVLGPGQSAAAAAGPGVLGPYGPGASAAAAAGQYGPGVLGPGQYGPGSSGPGVLGPYGPGSSAAAAAGQYGPGVLGPYGPGQSAAAAAGQYVLGPGVLGPYGPGASGPGVLGPYGPGASAAAAAGPGQYGPGVLGPSASAAAAAGQYGSGPGQYGPYGPGQSGPGSGVLGQGPYGPGASAAAAAGQYGPGVLGPYGPGQSAAAAAGPGSGQYGPGASGQNGPGSGQYGPGVLGPGQSAAAAAGQYVLGPGVLGPYGPGASAAAAAGQYGSGPGVLGPYGPGQSGSGVLGPGVLGPYASAAAAAGPGSGVLGPGAS

SEQ ID NO: 28 - protein, 590 aa, Artificial Sequence
  M_PRT965
MGPGTSGPYGPGASAAAAAGANGPGSGTSGPGASGAYGPGTSGPGTSGPGSSAAAAAGPGAYGPGTSGPSASAAAAAGPGSGTSGPGASGAYGPGTSGPGTSGPGSSAAAAAGAYGSGPGTSGPYGSAAAAAGPGSGAYGAGPYGPGASGPGAYGPGTSGPSASAAAAAGSGTSGPGAYGPYASAAAAAGAYGSGPGTSGPYGPGASGSGTSGPGTSGPYASAAAAAGPGTSGPYGPGSSAAAAAGAYGYGPGTSGPYGPGASGANGPGSGAYGPGTSGPGASAAAAAGPGTSGPYGPGASAAAAAGAYGPGTSGPGAYGPGSSGPGTSGPYGPGSSAAAAAGAYGPGTSGPYGPGASAAAAAGAYTSGPGTSGPYGPGASGPGTSGPYGPGASAAAAAGPGAYGPGTSGPSASAAAAAGAYGSGPGAYGPYGPGASGPGSGTSGAGPYGPGASAAAAAGAYGPGTSGPYGPGASAAAAAGPGSGAYGPGASGANGPGSGAYGPGTSGPGASAAAAAGAYTSGPGTSGPYGPGASAAAAAGAYGSGPGTSGPYGPGASGSGTSGPGTSGPYASAAAAAGPGSGTSGPGAS

SEQ ID NO: 29 - protein, 593 aa, Artificial Sequence
  M_PRT889
MGSSGPGVLGPYGPGASAAAAAGINGPGSGVLGPGISGIYGPGVLGPGVLGPGSSAAAAAGPGIYGPGVLGPSASAAAAAGPGSGVLGPGASGIYGPGVLGPGVLGPGSSAAAAAGIYGSGPGVLGPYGSAAAAAGPGSGIYGIGPYGPGASGPGIYGPGVLGPSASAAAAAGSGVLGPGIYGPYASAAAAAGIYGSGPGVLGPYGPGISGSGVLGPGVLGPYASAAAAAGPGVLGPYGPGSSAAAAAGIYGYGPGVLGPYGPGASGINGPGSGIYGPGVLGPGISAAAAAGPGVLGPYGPGASAAAAAGIYGPGVLGPGIYGPGSSGPGVLGPYGPGSSAAAAAGIYGPGVLGPYGPGISAAAAAGIYVLGPGVLGPYGPGASGPGVLGPYGPGASAAAAAGPGIYGPGVLGPSASAAAAAGIYGSGPGIYGPYGPGISGPGSGVLGIGPYGPGASAAAAAGIYGPGVLGPYGPGISAAAAAGPGSGIYGPGASGINGPGSGIYGPGVLGPGISAAAAAGIYVLGPGVLGPYGPGASAAAAAGIYGSGPGVLGPYGPGISGSGVLGPGVLGPYASAAAAAGPGSGVLGPGAS

SEQ ID NO: 30 - protein, 590 aa, Artificial Sequence
  M_PRT916
MGPGVIGPYGPGASAAAAAGLNGPGSGVIGPGLSGLYGPGVIGPGVIGPGSSAAAAAGPGLYGPGVIGPSASAAAAAGPGSGVIGPGASGLYGPGVIGPGVIGPGSSAAAAAGLYGSGPGVIGPYGSAAAAAGPGSGLYGLGPYGPGASGPGLYGPGVIGPSASAAAAAGSGVIGPGLYGPYASAAAAAGLYGSGPGVIGPYGPGLSGSGVIGPGVIGPYASAAAAAGPGVIGPYGPGSSAAAAAGLYGYGPGVIGPYGPGASGLNGPGSGLYGPGVIGPGLSAAAAAGPGVIGPYGPGASAAAAAGLYGPGVIGPGLYGPGSSGPGVIGPYGPGSSAAAAAGLYGPGVIGPYGPGLSAAAAAGLYVIGPGVIGPYGPGASGPGVIGPYGPGASAAAAAGPGLYGPGVIGPSASAAAAAGLYGSGPGLYGPYGPGLSGPGSGVIGLGPYGPGASAAAAAGLYGPGVIGPYGPGLSAAAAAGPGSGLYGPGASGLNGPGSGLYGPGVIGPGLSAAAAAGLYVIGPGVIGPYGPGASAAAAAGLYGSGPGVIGPYGPGLSGSGVIGPGVIGPYASAAAAAGPGSGVIGPGAS

SEQ ID NO: 31 - protein, 590 aa, Artificial Sequence
  M_ PRT918
MGPGVFGPYGPGASAAAAAGINGPGSGVFGPGISGIYGPGVFGPGVFGPGSSAAAAAGPGIYGPGVFGPSASAAAAAGPGSGVFGPGASGIYGPGVFGPGVFGPGSSAAAAAGIYGSGPGVFGPYGSAAAAAGPGSGIYGIGPYGPGASGPGIYGPGVFGPSASAAAAAGSGVFGPGIYGPYASAAAAAGIYGSGPGVFGPYGPGISGSGVFGPGVFGPYASAAAAAGPGVFGPYGPGSSAAAAAGIYGYGPGVFGPYGPGASGINGPGSGIYGPGVFGPGISAAAAAGPGVFGPYGPGASAAAAAGIYGPGVFGPGIYGPGSSGPGVFGPYGPGSSAAAAAGIYGPGVFGPYGPGISAAAAAGIYVFGPGVFGPYGPGASGPGVFGPYGPGASAAAAAGPGIYGPGVFGPSASAAAAAGIYGSGPGIYGPYGPGISGPGSGVFGIGPYGPGASAAAAAGIYGPGVFGPYGPGISAAAAAGPGSGIYGPGASGINGPGSGIYGPGVFGPGISAAAAAGIYVFGPGVFGPYGPGASAAAAAGIYGSGPGVFGPYGPGISGSGVFGPGVFGPYASAAAAAGPGSGVFGPGAS

SEQ ID NO: 32 - protein, 565 aa, Artificial Sequence
  M_PRT699
MGPGVLGPYGPGASAAAAAAAGSNGPGSGVLGPGQSGQYGPGVLGPGVLGPGSSAAAAAAAGPGQYGPGVLGPSASAAAAAAAGPGSGVLGPGASGQYGPGVLGPGVLGPGSSAAAAAAAGSYGSGPGVLGPYGSAAAAAAAGPGSGQYGQGPYGPGASGPGQYGPGVLGPSASAAAAAAAGSGVLGPGQYGPYASAAAAAAAGSYGSGPGVLGPYGPGQSGSGVLGPGVLGPYASAAAAAAAGPGVLGPYGPGSSAAAAAAAGSYGYGPGVLGPYGPGASGQNGPGSGQYGPGVLGPGPSAAAAAAAGPGVLGPYGPGASAAAAAAAGSYGPGVLGPGQYGPGSSGPGVLGPYGPGSSAAAAAAAGSYGPGVLGPYGPGPSAAAAAAAGSYVLGPGVLGPYGPGASGPGVLGPYGPGASAAAAAAAGPGQYGPGVLGPSASAAAAAAAGSYGSGPGQYGPYGPGQSGPGSGVLGQGPYGPGASAAAAAAAGSYGPGVLGPYGPGPSAAAAAAAGPGSGQYGPGASGQNGPGSGQYGPGVLGPGPSAAAAAAAGPGSGVLGPGAS

SEQ ID NO: 33 - protein, 565 aa, Artificial Sequence
  M_PRT698
MGPGVLGPYGPGASAAAAAAAGSNGPGSGVLGPGISGIYGPGVLGPGVLGPGSSAAAAAAAGPGIYGPGVLGPSASAAAAAAAGPGSGVLGPGASGIYGPGVLGPGVLGPGSSAAAAAAAGSYGSGPGVLGPYGSAAAAAAAGPGSGIYGIGPYGPGASGPGIYGPGVLGPSASAAAAAAAGSGVLGPGIYGPYASAAAAAAAGSYGSGPGVLGPYGPGISGSGVLGPGVLGPYASAAAAAAAGPGVLGPYGPGSSAAAAAAAGSYGYGPGVLGPYGPGASGINGPGSGIYGPGVLGPGPSAAAAAAAGPGVLGPYGPGASAAAAAAAGSYGPGVLGPGIYGPGSSGPGVLGPYGPGSSAAAAAAAGSYGPGVLGPYGPGPSAAAAAAAGSYVLGPGVLGPYGPGASGPGVLGPYGPGASAAAAAAAGPGIYGPGVLGPSASAAAAAAAGSYGSGPGIYGPYGPGISGPGSGVLGIGPYGPGASAAAAAAAGSYGPGVLGPYGPGPSAAAAAAAGPGSGIYGPGASGINGPGSGIYGPGVLGPGPSAAAAAAAGPGSGVLGPGAS

SEQ ID NO: 34 - protein, 565 aa, Artificial Sequence; identical to SEQ ID NO: 8
  M_PRT525

SEQ ID NO: 35 - protein, 601 aa, Artificial Sequence
  PRT888
MHHHHHHSSGSSGPGVLGPYGPGASAAAAAGQNGPGSGVLGPGQSGQYGPGVLGPGVLGPGSSAAAAAGPGQYGPGVLGPSASAAAAAGPGSGVLGPGASGQYGPGVLGPGVLGPGSSAAAAAGQYGSGPGVLGPYGSAAAAAGPGSGQYGQGPYGPGASGPGQYGPGVLGPSASAAAAAGSGVLGPGQYGPYASAAAAAGQYGSGPGVLGPYGPGQSGSGVLGPGVLGPYASAAAAAGPGVLGPYGPGSSAAAAAGQYGYGPGVLGPYGPGASGQNGPGSGQYGPGVLGPGQSAAAAAGPGVLGPYGPGASAAAAAGQYGPGVLGPGQYGPGSSGPGVLGPYGPGSSAAAAAGQYGPGVLGPYGPGQSAAAAAGQYVLGPGVLGPYGPGASGPGVLGPYGPGASAAAAAGPGQYGPGVLGPSASAAAAAGQYGSGPGQYGPYGPGQSGPGSGVLGQGPYGPGASAAAAAGQYGPGVLGPYGPGQSAAAAAGPGSGQYGPGASGQNGPGSGQYGPGVLGPGQSAAAAAGQYVLGPGVLGPYGPGASAAAAAGQYGSGPGVLGPYGPGQSGSGVLGPGVLGPYASAAAAAGPGSGVLGPGAS

SEQ ID NO: 36 - protein, 601 aa, Artificial Sequence
  PRT965
MHHHHHHSSGSSGPGTSGPYGPGASAAAAAGANGPGSGTSGPGASGAYGPGTSGPGTSGPGSSAAAAAGPGAYGPGTSGPSASAAAAAGPGSGTSGPGASGAYGPGTSGPGTSGPGSSAAAAAGAYGSGPGTSGPYGSAAAAAGPGSGAYGAGPYGPGASGPGAYGPGTSGPSASAAAAAGSGTSGPGAYGPYASAAAAAGAYGSGPGTSGPYGPGASGSGTSGPGTSGPYASAAAAAGPGTSGPYGPGSSAAAAAGAYGYGPGTSGPYGPGASGANGPGSGAYGPGTSGPGASAAAAAGPGTSGPYGPGASAAAAAGAYGPGTSGPGAYGPGSSGPGTSGPYGPGSSAAAAAGAYGPGTSGPYGPGASAAAAAGAYTSGPGTSGPYGPGASGPGTSGPYGPGASAAAAAGPGAYGPGTSGPSASAAAAAGAYGSGPGAYGPYGPGASGPGSGTSGAGPYGPGASAAAAAGAYGPGTSGPYGPGASAAAAAGPGSGAYGPGASGANGPGSGAYGPGTSGPGASAAAAAGAYTSGPGTSGPYGPGASAAAAAGAYGSGPGTSGPYGPGASGSGTSGPGTSGPYASAAAAAGPGSGTSGPGAS

SEQ ID NO: 37 - protein, 601 aa, Artificial Sequence
  PRT889
MHHHHHHSSGSSGPGVLGPYGPGASAAAAAGINGPGSGVLGPGISGIYGPGVLGPGVLGPGSSAAAAAGPGIYGPGVLGPSASAAAAAGPGSGVLGPGASGIYGPGVLGPGVLGPGSSAAAAAGIYGSGPGVLGPYGSAAAAAGPGSGIYGIGPYGPGASGPGIYGPGVLGPSASAAAAAGSGVLGPGIYGPYASAAAAAGIYGSGPGVLGPYGPGISGSGVLGPGVLGPYASAAAAAGPGVLGPYGPGSSAAAAAGIYGYGPGVLGPYGPGASGINGPGSGIYGPGVLGPGISAAAAAGPGVLGPYGPGASAAAAAGIYGPGVLGPGIYGPGSSGPGVLGPYGPGSSAAAAAGIYGPGVLGPYGPGISAAAAAGIYVLGPGVLGPYGPGASGPGVLGPYGPGASAAAAAGPGIYGPGVLGPSASAAAAAGIYGSGPGIYGPYGPGISGPGSGVLGIGPYGPGASAAAAAGIYGPGVLGPYGPGISAAAAAGPGSGIYGPGASGINGPGSGIYGPGVLGPGISAAAAAGIYVLGPGVLGPYGPGASAAAAAGIYGSGPGVLGPYGPGISGSGVLGPGVLGPYASAAAAAGPGSGVLGPGAS

SEQ ID NO: 38 - protein, 601 aa, Artificial Sequence
  PRT916
MHHHHHHSSGSSGPGVIGPYGPGASAAAAAGLNGPGSGVIGPGLSGLYGPGVIGPGVIGPGSSAAAAAGPGLYGPGVIGPSASAAAAAGPGSGVIGPGASGLYGPGVIGPGVIGPGSSAAAAAGLYGSGPGVIGPYGSAAAAAGPGSGLYGLGPYGPGASGPGLYGPGVIGPSASAAAAAGSGVIGPGLYGPYASAAAAAGLYGSGPGVIGPYGPGLSGSGVIGPGVIGPYASAAAAAGPGVIGPYGPGSSAAAAAGLYGYGPGVIGPYGPGASGLNGPGSGLYGPGVIGPGLSAAAAAGPGVIGPYGPGASAAAAAGLYGPGVIGPGLYGPGSSGPGVIGPYGPGSSAAAAAGLYGPGVIGPYGPGLSAAAAAGLYVIGPGVIGPYGPGASGPGVIGPYGPGASAAAAAGPGLYGPGVIGPSASAAAAAGLYGSGPGLYGPYGPGLSGPGSGVIGLGPYGPGASAAAAAGLYGPGVIGPYGPGLSAAAAAGPGSGLYGPGASGLNGPGSGLYGPGVIGPGLSAAAAAGLYVIGPGVIGPYGPGASAAAAAGLYGSGPGVIGPYGPGLSGSGVIGPGVIGPYASAAAAAGPGSGVIGPGAS

SEQ ID NO: 39 - protein, 601 aa, Artificial Sequence
  PRT918
MHHHHHHSSGSSGPGVFGPYGPGASAAAAAGINGPGSGVFGPGISGIYGPGVFGPGVFGPGSSAAAAAGPGIYGPGVFGPSASAAAAAGPGSGVFGPGASGIYGPGVFGPGVFGPGSSAAAAAGIYGSGPGVFGPYGSAAAAAGPGSGIYGIGPYGPGASGPGIYGPGVFGPSASAAAAAGSGVFGPGIYGPYASAAAAAGIYGSGPGVFGPYGPGISGSGVFGPGVFGPYASAAAAAGPGVFGPYGPGSSAAAAAGIYGYGPGVFGPYGPGASGINGPGSGIYGPGVFGPGISAAAAAGPGVFGPYGPGASAAAAAGIYGPGVFGPGIYGPGSSGPGVFGPYGPGSSAAAAAGIYGPGVFGPYGPGISAAAAAGIYVFGPGVFGPYGPGASGPGVFGPYGPGASAAAAAGPGIYGPGVFGPSASAAAAAGIYGSGPGIYGPYGPGISGPGSGVFGIGPYGPGASAAAAAGIYGPGVFGPYGPGISAAAAAGPGSGIYGPGASGINGPGSGIYGPGVFGPGISAAAAAGIYVFGPGVFGPYGPGASAAAAAGIYGSGPGVFGPYGPGISGSGVFGPGVFGPYASAAAAAGPGSGVFGPGAS

SEQ ID NO: 40 - protein, 576 aa, Artificial Sequence
  PRT699
MHHHHHHSSGSSGPGVLGPYGPGASAAAAAAAGSNGPGSGVLGPGQSGQYGPGVLGPGVLGPGSSAAAAAAAGPGQYGPGVLGPSASAAAAAAAGPGSGVLGPGASGQYGPGVLGPGVLGPGSSAAAAAAAGSYGSGPGVLGPYGSAAAAAAAGPGSGQYGQGPYGPGASGPGQYGPGVLGPSASAAAAAAAGSGVLGPGQYGPYASAAAAAAAGSYGSGPGVLGPYGPGQSGSGVLGPGVLGPYASAAAAAAAGPGVLGPYGPGSSAAAAAAAGSYGYGPGVLGPYGPGASGQNGPGSGQYGPGVLGPGPSAAAAAAAGPGVLGPYGPGASAAAAAAAGSYGPGVLGPGQYGPGSSGPGVLGPYGPGSSAAAAAAAGSYGPGVLGPYGPGPSAAAAAAAGSYVLGPGVLGPYGPGASGPGVLGPYGPGASAAAAAAAGPGQYGPGVLGPSASAAAAAAAGSYGSGPGQYGPYGPGQSGPGSGVLGQGPYGPGASAAAAAAAGSYGPGVLGPYGPGPSAAAAAAAGPGSGQYGPGASGQNGPGSGQYGPGVLGPGPSAAAAAAAGPGSGVLGPGAS

SEQ ID NO: 41 - protein, 576 aa, Artificial Sequence
  PRT698
MHHHHHHSSGSSGPGVLGPYGPGASAAAAAAAGSNGPGSGVLGPGISGIYGPGVLGPGVLGPGSSAAAAAAAGPGIYGPGVLGPSASAAAAAAAGPGSGVLGPGASGIYGPGVLGPGVLGPGSSAAAAAAAGSYGSGPGVLGPYGSAAAAAAAGPGSGIYGIGPYGPGASGPGIYGPGVLGPSASAAAAAAAGSGVLGPGIYGPYASAAAAAAAGSYGSGPGVLGPYGPGISGSGVLGPGVLGPYASAAAAAAAGPGVLGPYGPGSSAAAAAAAGSYGYGPGVLGPYGPGASGINGPGSGIYGPGVLGPGPSAAAAAAAGPGVLGPYGPGASAAAAAAAGSYGPGVLGPGIYGPGSSGPGVLGPYGPGSSAAAAAAAGSYGPGVLGPYGPGPSAAAAAAAGSYVLGPGVLGPYGPGASGPGVLGPYGPGASAAAAAAAGPGIYGPGVLGPSASAAAAAAAGSYGSGPGIYGPYGPGISGPGSGVLGIGPYGPGASAAAAAAAGSYGPGVLGPYGPGPSAAAAAAAGPGSGIYGPGASGINGPGSGIYGPGVLGPGPSAAAAAAAGPGSGVLGPGAS

SEQ ID NO: 42 - protein, 17 aa, Artificial Sequence
  Hinge+His-tag
SSVDKLAAALEHHHHHH

SEQ ID NO: 43 - protein, 1179 aa, Artificial Sequence
  Met-PRT966
MGPGVFGPYGPGASAAAAAGINGPGSGVFGPGISGIYGPGVFGPGVFGPGSSAAAAAGPGIYGPGVFGPSASAAAAAGPGSGVFGPGASGIYGPGVFGPGVFGPGSSAAAAAGIYGSGPGVFGPYGSAAAAAGPGSGIYGIGPYGPGASGPGIYGPGVFGPSASAAAAAGSGVFGPGIYGPYASAAAAAGIYGSGPGVFGPYGPGISGSGVFGPGVFGPYASAAAAAGPGVFGPYGPGSSAAAAAGIYGYGPGVFGPYGPGASGINGPGSGIYGPGVFGPGISAAAAAGPGVFGPYGPGASAAAAAGIYGPGVFGPGIYGPGSSGPGVFGPYGPGSSAAAAAGIYGPGVFGPYGPGISAAAAAGIYVFGPGVFGPYGPGASGPGVFGPYGPGASAAAAAGPGIYGPGVFGPSASAAAAAGIYGSGPGIYGPYGPGISGPGSGVFGIGPYGPGASAAAAAGIYGPGVFGPYGPGISAAAAAGPGSGIYGPGASGINGPGSGIYGPGVFGPGISAAAAAGIYVFGPGVFGPYGPGASAAAAAGIYGSGPGVFGPYGPGISGSGVFGPGVFGPYASAAAAAGPGSGVFGPGASGPGVFGPYGPGASAAAAAGINGPGSGVFGPGISGIYGPGVFGPGVFGPGSSAAAAAGPGIYGPGVFGPSASAAAAAGPGSGVFGPGASGIYGPGVFGPGVFGPGSSAAAAAGIYGSGPGVFGPYGSAAAAAGPGSGIYGIGPYGPGASGPGIYGPGVFGPSASAAAAAGSGVFGPGIYGPYASAAAAAGIYGSGPGVFGPYGPGISGSGVFGPGVFGPYASAAAAAGPGVFGPYGPGSSAAAAAGIYGYGPGVFGPYGPGASGINGPGSGIYGPGVFGPGISAAAAAGPGVFGPYGPGASAAAAAGIYGPGVFGPGIYGPGSSGPGVFGPYGPGSSAAAAAGIYGPGVFGPYGPGISAAAAAGIYVFGPGVFGPYGPGASGPGVFGPYGPGASAAAAAGPGIYGPGVFGPSASAAAAAGIYGSGPGIYGPYGPGISGPGSGVFGIGPYGPGASAAAAAGIYGPGVFGPYGPGISAAAAAGPGSGIYGPGASGINGPGSGIYGPGVFGPGISAAAAAGIYVFGPGVFGPYGPGASAAAAAGIYGSGPGVFGPYGPGISGSGVFGPGVFGPYASAAAAAGPGSGVFGPGAS

SEQ ID NO: 44 - protein, 1190 aa, Artificial Sequence
  PRT966
MHHHHHHSSGSSGPGVFGPYGPGASAAAAAGINGPGSGVFGPGISGIYGPGVFGPGVFGPGSSAAAAAGPGIYGPGVFGPSASAAAAAGPGSGVFGPGASGIYGPGVFGPGVFGPGSSAAAAAGIYGSGPGVFGPYGSAAAAAGPGSGIYGIGPYGPGASGPGIYGPGVFGPSASAAAAAGSGVFGPGIYGPYASAAAAAGIYGSGPGVFGPYGPGISGSGVFGPGVFGPYASAAAAAGPGVFGPYGPGSSAAAAAGIYGYGPGVFGPYGPGASGINGPGSGIYGPGVFGPGISAAAAAGPGVFGPYGPGASAAAAAGIYGPGVFGPGIYGPGSSGPGVFGPYGPGSSAAAAAGIYGPGVFGPYGPGISAAAAAGIYVFGPGVFGPYGPGASGPGVFGPYGPGASAAAAAGPGIYGPGVFGPSASAAAAAGIYGSGPGIYGPYGPGISGPGSGVFGIGPYGPGASAAAAAGIYGPGVFGPYGPGISAAAAAGPGSGIYGPGASGINGPGSGIYGPGVFGPGISAAAAAGIYVFGPGVFGPYGPGASAAAAAGIYGSGPGVFGPYGPGISGSGVFGPGVFGPYASAAAAAGPGSGVFGPGASGPGVFGPYGPGASAAAAAGINGPGSGVFGPGISGIYGPGVFGPGVFGPGSSAAAAAGPGIYGPGVFGPSASAAAAAGPGSGVFGPGASGIYGPGVFGPGVFGPGSSAAAAAGIYGSGPGVFGPYGSAAAAAGPGSGIYGIGPYGPGASGPGIYGPGVFGPSASAAAAAGSGVFGPGIYGPYASAAAAAGIYGSGPGVFGPYGPGISGSGVFGPGVFGPYASAAAAAGPGVFGPYGPGSSAAAAAGIYGYGPGVFGPYGPGASGINGPGSGIYGPGVFGPGISAAAAAGPGVFGPYGPGASAAAAAGIYGPGVFGPGIYGPGSSGPGVFGPYGPGSSAAAAAGIYGPGVFGPYGPGISAAAAAGIYVFGPGVFGPYGPGASGPGVFGPYGPGASAAAAAGPGIYGPGVFGPSASAAAAAGIYGSGPGIYGPYGPGISGPGSGVFGIGPYGPGASAAAAAGIYGPGVFGPYGPGISAAAAAGPGSGIYGPGASGINGPGSGIYGPGVFGPGISAAAAAGIYVFGPGVFGPYGPGASAAAAAGIYGSGPGVFGPYGPGISGSGVFGPGVFGPYASAAAAAGPGSGVFGPGAS

SEQ ID NO: 45 - protein, 252 aa, Artificial Sequence
  Collagen-type4-Kai
MHHHHHHSSGSSKDGVPGFPGSEGVKGNRGFPGLMGEDGIKGQKGDIGPPGFRGPTEYYDTYQEKGDEGTPGPPGPRGARGPQGPSGPPGVPGSPGSSRPGLRGAPGWPGLKGSKGERGRPGKDAMGTPGSPGCAGSPGLPGSPGPPGPPGDIVFRKGPPGDHGLPGYLGSPGIPGVDGPKGEPGLLCTQCPYIPGPPGLPGLPGLHGVKGIPGRQGAAGLKGSPGSPGNTGLPGFPGFPGAQGDPGLKGEK

SEQ ID NO: 46 - protein, 12 aa, Artificial Sequence
  HisTag
MHHHHHHSSGSS

SEQ ID NO: 47 - protein, 310 aa, Artificial Sequence
  Resilin-Kai
MHHHHHHPEPPVNSYLPPSDSYGAPGQSGPGGRPSDSYGAPGGGNGGRPSDSYGAPGQGQGQGQGQGGYAGKPSDSYGAPGGGDGNGGRPSSSYGAPGGGNGGRPSDTYGAPGGGNGGRPSDTYGAPGGGGNGNGGRPSSSYGAPGQGQGNGNGGRPSSSYGAPGGGNGGRPSDTYGAPGGGNGGRPSDTYGAPGGGNNGGRPSSSYGAPGGGNGGRPSDTYGAPGGGNGNGSGGRPSSSYGAPGQGQGGFGGRPSDSYGAPGQNQKPSDSYGAPGSGNGNGGRPSSSYGAPGSGPGGRPSDSYGPPASG

SEQ ID NO: 48 - protein, 282 aa, Artificial Sequence
  elastin short
MHHHHHHSSGSSLGVSAGAVVPQPGAGVKPGKVPGVGLPGVYPGGVLPGARFPGVGVLPGVPTGAGVKPKAPGVGGAFAGIPGVGPFGGPQPGVPLGYPIKAPKLPGGYGLPYTTGKLPYGYGPGGVAGAAGKAGYPTGTGVGPQAAAAAAAKAAAKFGAGAAGVLPGVGGAGVPGVPGAIPGIGGIAGVGTPAAAAAAAAAAKAAKYGAAAGLVPGGPGFGPGVVGVPGAGVPGVGVPGAGIPVVPGAGIPGAAVPGVVSPEAAAKAAAKAAKYGARPGVG

SEQ ID NO: 49 - protein, 535 aa, Artificial Sequence
  type I keratin 26
MSFRLSGVSRRLCSQAGTGRLTGGRTGFRAGNVCSGLGAGSSFSGPLGSVSSKGSFSHGGGGLGSGVCTGFLENEHGLLPGNEKVTLQNLNDRLASYLDHVCTLEEANADLEQKIKGWYEKYGPGSGRQLAHDYSKYFSVTEDLKRQIISVTTCNASIVLQNENARLTADDFRLKCENELALHQSVEADINGLHRVMDELTLCTSDLEMQCEALSEELTYLKKNHQEEMKVMQGAARGNVLKCENELALHQSVEADINGLHRVMDELTLCTSDLEMQCEALSEELTYLKKNHQEEMKVMQGAARGNVNVEINAAPGVDLTVLLNNMRAEYEDLAEQNHEDAEAWFSEKSTSLHQQISDDAGAAMAARNELMELKRNLQTLEIELQSLLAMKHSYECSLAETESNYCHQLQQIQEQIGAMEDQLQQIRMETEGQKLEHERLLDVKIFLEKEIEMYCKLIDGEGRKSKSTCYKSEGRGPKNSENQVKDSKEEAVVKTVVGELDQLGSVLSLRVHSVEEKSSKISNITMEQRLPSKVP

SEQ ID NO: 50 - protein, 2268 aa, Artificial Sequence
  PRT705
MHHHHHHSSGSSGPGQQGPYGPGASAAAAAAAGSNGPGSGQQGPGQSGQYGPGQQGPGQQGPGSSAAAAAAAGPGQYGPGQQGPSASAAAAAAAGPGSGQQGPGASGQYGPGQQGPGQQGPGSSAAAAAAAGSYGSGPGQQGPYGSAAAAAAAGPGSGQYGQGPYGPGASGPGQYGPGQQGPSASAAAAAAAGSGQQGPGQYGPYASAAAAAAAGSYGSGPGQQGPYGPGQSGSGQQGPGQQGPYASAAAAAAAGPGQQGPYGPGSSAAAAAAAGSYGYGPGQQGPYGPGASGQNGPGSGQYGPGQQGPGPSAAAAAAAGPGQQGPYGPGASAAAAAAAGSYGPGQQGPGQYGPGSSGPGQQGPYGPGSSAAAAAAAGSYGPGQQGPYGPGPSAAAAAAAGSYQQGPGQQGPYGPGASGPGQQGPYGPGASAAAAAAAGPGQYGPGQQGPSASAAAAAAAGSYGSGPGQYGPYGPGQSGPGSGQQGQGPYGPGASAAAAAAAGSYGPGQQGPYGPGPSAAAAAAAGPGSGQYGPGASGQNGPGSGQYGPGQQGPGPSAAAAAAAGPGSGQQGPGASGQQGPYGPGASAAAAAAAGSNGPGSGQQGPGQSGQYGPGQQGPGQQGPGSSAAAAAAAGPGQYGPGQQGPSASAAAAAAAGPGSGQQGPGASGQYGPGQQGPGQQGPGSSAAAAAAAGSYGSGPGQQGPYGSAAAAAAAGPGSGQYGQGPYGPGASGPGQYGPGQQGPSASAAAAAAAGSGQQGPGQYGPYASAAAAAAAGSYGSGPGQQGPYGPGQSGSGQQGPGQQGPYASAAAAAAAGPGQQGPYGPGSSAAAAAAAGSYGYGPGQQGPYGPGASGQNGPGSGQYGPGQQGPGPSAAAAAAAGPGQQGPYGPGASAAAAAAAGSYGPGQQGPGQYGPGSSGPGQQGPYGPGSSAAAAAAAGSYGPGQQGPYGPGPSAAAAAAAGSYQQGPGQQGPYGPGASGPGQQGPYGPGASAAAAAAAGPGQYGPGQQGPSASAAAAAAAGSYGSGPGQYGPYGPGQSGPGSGQQGQGPYGPGASAAAAAAAGSYGPGQQGPYGPGPSAAAAAAAGPGSGQYGPGASGQNGPGSGQYGPGQQGPGPSAAAAAAAGPGSGQQGPGASEFELVDGQQGPYGPGASAAAAAAAGSNGPGSGQQGPGQSGQYGPGQQGPGQQGPGSSAAAAAAAGPGQYGPGQQGPSASAAAAAAAGPGSGQQGPGASGQYGPGQQGPGQQGPGSSAAAAAAAGSYGSGPGQQGPYGSAAAAAAAGPGSGQYGQGPYGPGASGPGQYGPGQQGPSASAAAAAAAGSGQQGPGQYGPYASAAAAAAAGSYGSGPGQQGPYGPGQSGSGQQGPGQQGPYASAAAAAAAGPGQQGPYGPGSSAAAAAAAGSYGYGPGQQGPYGPGASGQNGPGSGQYGPGQQGPGPSAAAAAAAGPGQQGPYGPGASAAAAAAAGSYGPGQQGPGQYGPGSSGPGQQGPYGPGSSAAAAAAAGSYGPGQQGPYGPGPSAAAAAAAGSYQQGPGQQGPYGPGASGPGQQGPYGPGASAAAAAAAGPGQYGPGQQGPSASAAAAAAAGSYGSGPGQYGPYGPGQSGPGSGQQGQGPYGPGASAAAAAAAGSYGPGQQGPYGPGPSAAAAAAAGPGSGQYGPGASGQNGPGSGQYGPGQQGPGPSAAAAAAAGPGSGQQGPGASGQQGPYGPGASAAAAAAAGSNGPGSGQQGPGQSGQYGPGQQGPGQQGPGSSAAAAAAAGPGQYGPGQQGPSASAAAAAAAGPGSGQQGPGASGQYGPGQQGPGQQGPGSSAAAAAAAGSYGSGPGQQGPYGSAAAAAAAGPGSGQYGQGPYGPGASGPGQYGPGQQGPSASAAAAAAAGSGQQGPGQYGPYASAAAAAAAGSYGSGPGQQGPYGPGQSGSGQQGPGQQGPYASAAAAAAAGPGQQGPYGPGSSAAAAAAAGSYGYGPGQQGPYGPGASGQNGPGSGQYGPGQQGPGPSAAAAAAAGPGQQGPYGPGASAAAAAAAGSYGPGQQGPGQYGPGSSGPGQQGPYGPGSSAAAAAAAGSYGPGQQGPYGPGPSAAAAAAAGSYQQGPGQQGPYGPGASGPGQQGPYGPGASAAAAAAAGPGQYGPGQQGPSASAAAAAAAGSYGSGPGQYGPYGPGQSGPGSGQQGQGPYGPGASAAAAAAAGSYGPGQQGPYGPGPSAAAAAAAGPGSGQYGPGASGQNGPGSGQYGPGQQGPGPSAAAAAAAGPGSGQQGPGAS

SEQ ID NO: 51 - protein, 601 aa, Artificial Sequence
  PRT826
MHHHHHHTTGTTGPGQQGPYGPGATAAAAAGQNGPGTGQQGPGQTGQYGPGQQGPGQQGPGTTAAAAAGPGQYGPGQQGPTATAAAAAGPGTGQQGPGATGQYGPGQQGPGQQGPGTTAAAAAGQYGTGPGQQGPYGTAAAAAGPGTGQYGQGPYGPGATGPGQYGPGQQGPTATAAAAAGTGQQGPGQYGPYATAAAAAGQYGTGPGQQGPYGPGQTGTGQQGPGQQGPYATAAAAAGPGQQGPYGPGTTAAAAAGQYGYGPGQQGPYGPGATGQNGPGTGQYGPGQQGPGQTAAAAAGPGQQGPYGPGATAAAAAGQYGPGQQGPGQYGPGTTGPGQQGPYGPGTTAAAAAGQYGPGQQGPYGPGQTAAAAAGQYQQGPGQQGPYGPGATGPGQQGPYGPGATAAAAAGPGQYGPGQQGPTATAAAAAGQYGTGPGQYGPYGPGQTGPGTGQQGQGPYGPGATAAAAAGQYGPGQQGPYGPGQTAAAAAGPGTGQYGPGATGQNGPGTGQYGPGQQGPGQTAAAAAGQYQQGPGQQGPYGPGATAAAAAGQYGTGPGQQGPYGPGQTGTGQQGPGQQGPYATAAAAAGPGTGQQGPGAT

SEQ ID NO: 52 - protein, 2476 aa, Artificial Sequence
  PRT853
MHHHHHHSSGSSGPGQQGPYGPGASAAAAAAGQNGPGSGQQGPGQSGQYGPGQQGPGQQGPGSSAAAAAAGPGQYGPGQQGPSASAAAAAAGPGSGQQGPGASGQYGPGQQGPGQQGPGSSAAAAAAGQYGSGPGQQGPYGSAAAAAAGPGSGQYGQGPYGPGASGPGQYGPGQQGPSASAAAAAAGSGQQGPGQYGPYASAAAAAAGQYGSGPGQQGPYGPGQSGSGQQGPGQQGPYASAAAAAAGPGQQGPYGPGSSAAAAAAGQYGYGPGQQGPYGPGASGQNGPGSGQYGPGQQGPGQSAAAAAAGPGQQGPYGPGASAAAAAAGQYGPGQQGPGQYGPGSSGPGQQGPYGPGSSAAAAAAGQYGPGQQGPYGPGQSAAAAAAGQYQQGPGQQGPYGPGASGPGQQGPYGPGASAAAAAAGPGQYGPGQQGPSASAAAAAAGQYGSGPGQYGPYGPGQSGPGSGQQGQGPYGPGASAAAAAAGQYGPGQQGPYGPGQSAAAAAAGPGSGQYGPGASGQNGPGSGQYGPGQQGPGQSAAAAAAGQYQQGPGQQGPYGPGASAAAAAAGQYGSGPGQQGPYGPGQSGSGQQGPGQQGPYASAAAAAAGPGSGQQGPGASAAAAAAAEFGQQGPYGPGASAAAAAAGQNGPGSGQQGPGQSGQYGPGQQGPGQQGPGSSAAAAAAGPGQYGPGQQGPSASAAAAAAGPGSGQQGPGASGQYGPGQQGPGQQGPGSSAAAAAAGQYGSGPGQQGPYGSAAAAAAGPGSGQYGQGPYGPGASGPGQYGPGQQGPSASAAAAAAGSGQQGPGQYGPYASAAAAAAGQYGSGPGQQGPYGPGQSGSGQQGPGQQGPYASAAAAAAGPGQQGPYGPGSSAAAAAAGQYGYGPGQQGPYGPGASGQNGPGSGQYGPGQQGPGQSAAAAAAGPGQQGPYGPGASAAAAAAGQYGPGQQGPGQYGPGSSGPGQQGPYGPGSSAAAAAAGQYGPGQQGPYGPGQSAAAAAAGQYQQGPGQQGPYGPGASGPGQQGPYGPGASAAAAAAGPGQYGPGQQGPSASAAAAAAGQYGSGPGQYGPYGPGQSGPGSGQQGQGPYGPGASAAAAAAGQYGPGQQGPYGPGQSAAAAAAGPGSGQYGPGASGQNGPGSGQYGPGQQGPGQSAAAAAAGQYQQGPGQQGPYGPGASAAAAAAGQYGSGPGQQGPYGPGQSGSGQQGPGQQGPYASAAAAAAGPGSGQQGPGASAAAAAAAELGQQGPYGPGASAAAAAAGQNGPGSGQQGPGQSGQYGPGQQGPGQQGPGSSAAAAAAGPGQYGPGQQGPSASAAAAAAGPGSGQQGPGASGQYGPGQQGPGQQGPGSSAAAAAAGQYGSGPGQQGPYGSAAAAAAGPGSGQYGQGPYGPGASGPGQYGPGQQGPSASAAAAAAGSGQQGPGQYGPYASAAAAAAGQYGSGPGQQGPYGPGQSGSGQQGPGQQGPYASAAAAAAGPGQQGPYGPGSSAAAAAAGQYGYGPGQQGPYGPGASGQNGPGSGQYGPGQQGPGQSAAAAAAGPGQQGPYGPGASAAAAAAGQYGPGQQGPGQYGPGSSGPGQQGPYGPGSSAAAAAAGQYGPGQQGPYGPGQSAAAAAAGQYQQGPGQQGPYGPGASGPGQQGPYGPGASAAAAAAGPGQYGPGQQGPSASAAAAAAGQYGSGPGQYGPYGPGQSGPGSGQQGQGPYGPGASAAAAAAGQYGPGQQGPYGPGQSAAAAAAGPGSGQYGPGASGQNGPGSGQYGPGQQGPGQSAAAAAAGQYQQGPGQQGPYGPGASAAAAAAGQYGSGPGQQGPYGPGQSGSGQQGPGQQGPYASAAAAAAGPGSGQQGPGASAAAAAAAKLGQQGPYGPGASAAAAAAGQNGPGSGQQGPGQSGQYGPGQQGPGQQGPGSSAAAAAAGPGQYGPGQQGPSASAAAAAAGPGSGQQGPGASGQYGPGQQGPGQQGPGSSAAAAAAGQYGSGPGQQGPYGSAAAAAAGPGSGQYGQGPYGPGASGPGQYGPGQQGPSASAAAAAAGSGQQGPGQYGPYASAAAAAAGQYGSGPGQQGPYGPGQSGSGQQGPGQQGPYASAAAAAAGPGQQGPYGPGSSAAAAAAGQYGYGPGQQGPYGPGASGQNGPGSGQYGPGQQGPGQSAAAAAAGPGQQGPYGPGASAAAAAAGQYGPGQQGPGQYGPGSSGPGQQGPYGPGSSAAAAAAGQYGPGQQGPYGPGQSAAAAAAGQYQQGPGQQGPYGPGASGPGQQGPYGPGASAAAAAAGPGQYGPGQQGPSASAAAAAAGQYGSGPGQYGPYGPGQSGPGSGQQGQGPYGPGASAAAAAAGQYGPGQQGPYGPGQSAAAAAAGPGSGQYGPGASGQNGPGSGQYGPGQQGPGQSAAAAAAGQYQQGPGQQGPYGPGASAAAAAAGQYGSGPGQQGPYGPGQSGSGQQGPGQQGPYASAAAAAAGPGSGQQGPGASAAAAAAA

SEQ ID NO: 53 - protein, 601 aa, Artificial Sequence
  PRT1103
MHHHHHHAAGAAGPGQQGPFGPGAGAAAAAGQNGPGAGQQGPGQAGQFGPGQQGPGQQGPGAGAAAAAGPGQFGPGQQGPSAGAAAAAGPGAGQQGPGAAGQFGPGQQGPGQQGPGAGAAAAAGQFGAGPGQQGPFGGAAAAAGPGAGQFGQGPFGPGAAGPGQFGPGQQGPSAGAAAAAGAGQQGPGQFGPFAGAAAAAGQFGAGPGQQGPFGPGQAGAGQQGPGQQGPFAGAAAAAGPGQQGPFGPGAGAAAAAGQFGFGPGQQGPFGPGAAGQNGPGAGQFGPGQQGPGQGAAAAAGPGQQGPFGPGAGAAAAAGQFGPGQQGPGQFGPGAAGPGQQGPFGPGAGAAAAAGQFGPGQQGPFGPGQGAAAAAGQFQQGPGQQGPFGPGAAGPGQQGPFGPGAGAAAAAGPGQFGPGQQGPSAGAAAAAGQFGAGPGQFGPFGPGQAGPGAGQQGQGPFGPGAGAAAAAGQFGPGQQGPFGPGQGAAAAAGPGAGQFGPGAAGQNGPGAGQFGPGQQGPGQGAAAAAGQFQQGPGQQGPFGPGAGAAAAAGQFGAGPGQQGPFGPGQAGAGQQGPGQQGPFAGAAAAAGPGAGQQGPGAS

SEQ ID NO: 54 - protein, 601 aa, Artificial Sequence
  PRT1104
MHHHHHHAAGAAGPGQQGPYGPGAGAAAAAGQNGPGAGQQGPGQAGQYGPGQQGPGQQGPGAGAAAAAGPGQYGPGQQGPSAGAAAAAGPGAGQQGPGAAGQYGPGQQGPGQQGPGAGAAAAAGQYGAGPGQQGPYGGAAAAAGPGAGQYGQGPYGPGAAGPGQYGPGQQGPSAGAAAAAGAGQQGPGQYGPYAGAAAAAGQYGAGPGQQGPYGPGQAGAGQQGPGQQGPYAGAAAAAGPGQQGPYGPGAGAAAAAGQYGYGPGQQGPYGPGAAGQNGPGAGQYGPGQQGPGQGAAAAAGPGQQGPYGPGAGAAAAAGQYGPGQQGPGQYGPGAAGPGQQGPYGPGAGAAAAAGQYGPGQQGPYGPGQGAAAAAGQYQQGPGQQGPYGPGAAGPGQQGPYGPGAGAAAAAGPGQYGPGQQGPSAGAAAAAGQYGAGPGQYGPYGPGQAGPGAGQQGQGPYGPGAGAAAAAGQYGPGQQGPYGPGQGAAAAAGPGAGQYGPGAAGQNGPGAGQYGPGQQGPGQGAAAAAGQYQQGPGQQGPYGPGAGAAAAAGQYGAGPGQQGPYGPGQAGAGQQGPGQQGPYAGAAAAAGPGAGQQGPGAS

SEQ ID NO: 55 - protein, 601 aa, Artificial Sequence
  PRT1107
MHHHHHHAAGAAGPGVFGPYGPGAVAAAAAGINGPGAGVFGPGILGIYGPGVFGPGVFGPGALAAAAAGPGIYGPGVFGPIAVAAAAAGPGAGVFGPGALGIYGPGVFGPGVFGPGALAAAAAGIYGAGPGVFGPYGLAAAAAGPGAGIYGIGPYGPGALGPGIYGPGVFGPIAVAAAAAGAGVFGPGIYGPYAVAAAAAGIYGAGPGVFGPYGPGILGAGVFGPGVFGPYAVAAAAAGPGVFGPYGPGALAAAAAGIYGYGPGVFGPYGPGALGINGPGAGIYGPGVFGPGILAAAAAGPGVFGPYGPGAVAAAAAGIYGPGVFGPGIYGPGALGPGVFGPYGPGALAAAAAGIYGPGVFGPYGPGILAAAAAGIYVFGPGVFGPYGPGALGPGVFGPYGPGAVAAAAAGPGIYGPGVFGPIAVAAAAAGIYGAGPGIYGPYGPGILGPGAGVFGIGPYGPGAVAAAAAGIYGPGVFGPYGPGILAAAAAGPGAGIYGPGALGINGPGAGIYGPGVFGPGILAAAAAGIYVFGPGVFGPYGPGAVAAAAAGIYGAGPGVFGPYGPGILGAGVFGPGVFGPYAVAAAAAGPGAGVFGPGAI

SEQ ID NO: 56 - protein, 601 aa, Artificial Sequence
  PRT1083
MHHHHHHSSGSSGLGVFGLYGTGASAAAAAGIAGTGSGVFGTGISGIYGLGVFGLGVFGTGSSAAAAAGTGIYGLGVFGLSASAAAAAGTGSGVFGTGASGIYGLGVFGLGVFGTGSSAAAAAGIYGSGLGVFGLYGSAAAAAGTGSGIYGIGLYGTGASGTGIYGLGVFGLSASAAAAAGSGVFGTGIYGLYASAAAAAGIYGSGLGVFGLYGTGISGSGVFGLGVFGLYASAAAAAGLGVFGLYGTGSSAAAAAGIYGYGLGVFGLYGTGASGIAGTGSGIYGLGVFGTGISAAAAAGLGVFGLYGTGASAAAAAGIYGLGVFGTGIYGTGSSGLGVFGLYGTGSSAAAAAGIYGLGVFGLYGTGISAAAAAGIYVFGLGVFGLYGTGASGLGVFGLYGTGASAAAAAGTGIYGLGVFGLSASAAAAAGIYGSGTGIYGLYGTGISGTGSGVFGIGLYGTGASAAAAAGIYGLGVFGLYGTGISAAAAAGTGSGIYGTGASGIAGTGSGIYGLGVFGTGISAAAAAGIYVFGLGVFGLYGTGASAAAAAGIYGSGLGVFGLYGTGISGSGVFGLGVFGLYASAAAAAGTGSGVFGTGAS

SEQ ID NO: 57 - protein, 2266 aa, Artificial Sequence
  PRT1125
MHHHHHHSSGSSGPGQQGPYGPGASAAAAAAAGSNGPGSGQQGPGQSGQYGPGQQGPGQQGPGSSAAAAAAAGPGQYGPGQQGPSASAAAAAAAGPGSGQQGPGASGQYGPGQQGPGQQGPGSSAAAAAAAGSYGSGPGQQGPYGSAAAAAAAGPGSGQYGQGPYGPGASGPGQYGPGQQGPSASAAAAAAAGSGQQGPGQYGPYASAAAAAAAGSYGSGPGQQGPYGPGQSGSGQQGPGQQGPYASAAAAAAAGPGQQGPYGPGSSAAAAAAAGSYGYGPGQQGPYGPGASGQNGPGSGQYGPGQQGPGPSAAAAAAAGPGQQGPYGPGASAAAAAAAGSYGPGQQGPGQYGPGSSGPGQQGPYGPGSSAAAAAAAGSYGPGQQGPYGPGPSAAAAAAAGSYQQGPGQQGPYGPGASGPGQQGPYGPGASAAAAAAAGPGQYGPGQQGPSASAAAAAAAGSYGSGPGQYGPYGPGQSGPGSGQQGQGPYGPGASAAAAAAAGSYGPGQQGPYGPGPSAAAAAAAGPGSGQYGPGASGQNGPGSGQYGPGQQGPGPSAAAAAAAGPGSGQQGPGASELGQQGPYGPGASAAAAAAAGSNGPGSGQQGPGQSGQYGPGQQGPGQQGPGSSAAAAAAAGPGQYGPGQQGPSASAAAAAAAGPGSGQQGPGASGQYGPGQQGPGQQGPGSSAAAAAAAGSYGSGPGQQGPYGSAAAAAAAGPGSGQYGQGPYGPGASGPGQYGPGQQGPSASAAAAAAAGSGQQGPGQYGPYASAAAAAAAGSYGSGPGQQGPYGPGQSGSGQQGPGQQGPYASAAAAAAAGPGQQGPYGPGSSAAAAAAAGSYGYGPGQQGPYGPGASGQNGPGSGQYGPGQQGPGPSAAAAAAAGPGQQGPYGPGASAAAAAAAGSYGPGQQGPGQYGPGSSGPGQQGPYGPGSSAAAAAAAGSYGPGQQGPYGPGPSAAAAAAAGSYQQGPGQQGPYGPGASGPGQQGPYGPGASAAAAAAAGPGQYGPGQQGPSASAAAAAAAGSYGSGPGQYGPYGPGQSGPGSGQQGQGPYGPGASAAAAAAAGSYGPGQQGPYGPGPSAAAAAAAGPGSGQYGPGASGQNGPGSGQYGPGQQGPGPSAAAAAAAGPGSGQQGPGASGPGQQGPYGPGASAAAAAAAGSNGPGSGQQGPGQSGQYGPGQQGPGQQGPGSSAAAAAAAGPGQYGPGQQGPSASAAAAAAAGPGSGQQGPGASGQYGPGQQGPGQQGPGSSAAAAAAAGSYGSGPGQQGPYGSAAAAAAAGPGSGQYGQGPYGPGASGPGQYGPGQQGPSASAAAAAAAGSGQQGPGQYGPYASAAAAAAAGSYGSGPGQQGPYGPGQSGSGQQGPGQQGPYASAAAAAAAGPGQQGPYGPGSSAAAAAAAGSYGYGPGQQGPYGPGASGQNGPGSGQYGPGQQGPGPSAAAAAAAGPGQQGPYGPGASAAAAAAAGSYGPGQQGPGQYGPGSSGPGQQGPYGPGSSAAAAAAAGSYGPGQQGPYGPGPSAAAAAAAGSYQQGPGQQGPYGPGASGPGQQGPYGPGASAAAAAAAGPGQYGPGQQGPSASAAAAAAAGSYGSGPGQYGPYGPGQSGPGSGQQGQGPYGPGASAAAAAAAGSYGPGQQGPYGPGPSAAAAAAAGPGSGQYGPGASGQNGPGSGQYGPGQQGPGPSAAAAAAAGPGSGQQGPGASGQQGPYGPGASAAAAAAAGSNGPGSGQQGPGQSGQYGPGQQGPGQQGPGSSAAAAAAAGPGQYGPGQQGPSASAAAAAAAGPGSGQQGPGASGQYGPGQQGPGQQGPGSSAAAAAAAGSYGSGPGQQGPYGSAAAAAAAGPGSGQYGQGPYGPGASGPGQYGPGQQGPSASAAAAAAAGSGQQGPGQYGPYASAAAAAAAGSYGSGPGQQGPYGPGQSGSGQQGPGQQGPYASAAAAAAAGPGQQGPYGPGSSAAAAAAAGSYGYGPGQQGPYGPGASGQNGPGSGQYGPGQQGPGPSAAAAAAAGPGQQGPYGPGASAAAAAAAGSYGPGQQGPGQYGPGSSGPGQQGPYGPGSSAAAAAAAGSYGPGQQGPYGPGPSAAAAAAAGSYQQGPGQQGPYGPGASGPGQQGPYGPGASAAAAAAAGPGQYGPGQQGPSASAAAAAAAGSYGSGPGQYGPYGPGQSGPGSGQQGQGPYGPGASAAAAAAAGSYGPGQQGPYGPGPSAAAAAAAGPGSGQYGPGASGQNGPGSGQYGPGQQGPGPSAAAAAAAGPGSGQQGPGAS

SEQ ID NO: 58 - protein, 560 aa, Artificial Sequence
  PRT855
MHHHHHHSSGSSGEGAFQGPSFRGSGASRGAAAAAGSQAGTGRGTGGRTGFRAGNGCSGAGAAAAAGSSFSGPGGSASSKGSFSHGGAAAAAGGAGSGGCTGFGENEHGAAAAAGGNEKATGQNANDRGAAAAAGYADHGCTGEEANAGAAAAAGQKIKGWYEKYGPGSGRQGAAAAAGDYSKYFSATEDAKRQSGTTCGAAAAAGAGQNENARATADDFRGKCENGAAAAAGHQSGEADINGAHRAMDEGGAAAAAGTSDGEMQCEAASEEGTGAAAAAGKNHQEEMKGSFRGSGASRGAAAAAGSQAGTGRGTGGRTGFRAGNGCSGAGAAAAAGSSFSGPGGSASSKGSFSHGGAAAAAGGAGSGGCTGFGENEHGAAAAAGGNEKATGQNANDRGAAAAAGYADHGCTGEEANAGAAAAAGQKIKGWYEKYGPGSGRQGAAAAAGDYSKYFSATEDAKRQSGTTCGAAAAAGAGQNENARATADDFRGKCENGAAAAAGHQSGEADINGAHRAMDEGGAAAAAGTSDGEMQCEAASEEGTGAAAAAGKNHQEEMKG

SEQ ID NO: 59 - protein, 252 aa, Artificial Sequence; identical to SEQ ID NO: 45
  PRT537

SEQ ID NO: 60 - protein, 310 aa, Artificial Sequence; identical to SEQ ID NO: 47
  PRT366

SEQ ID NO: 61 - protein, 150 aa, Artificial Sequence
  PRT662
MHHHHHHQDPYVKEAENLKKYFNAGHSDVADNGTLFLGILKNWKEESDRKIMQSQIVSFYFKLFKNFKDDQSIQKSVETIKEDMNVKFFNSNKKKRDDFEKLTNYSVTDLNVQRKAIHELIQVMAELSPAAKTGKRKRSQMLFRGRRASQ

SEQ ID NO: 62 - protein, 7 aa, Artificial Sequence
  Amino acid sequence
GAAAAAG